European Patent Specification EP 3 770 271 B1, published February 8, 2023. Title: Targeted enrichment of long nucleotide sequences using microfluidic partitioning. Applicant: Samplix ApS. The sequence listing filed with the application follows.

SEQUENCE LISTING (24 sequences)

SEQ ID NO: 1 - DNA, 22 bp, Escherichia coli
  primer_bind (1)..(22): MB8 Fw1 tm60 primer for E. coli thrA
gacggtagattcgaggtaatgc

SEQ ID NO: 2 - DNA, 20 bp, Escherichia coli
  primer_bind (1)..(20): MB8 Rev1 tm60 primer for E. coli thrA
tatggccggcgtattagaag

SEQ ID NO: 3 - DNA, 18 bp, Escherichia coli
  primer_bind (1)..(18): MB10.1fw qPCR primer
tcaacaacctcgcatcgg

SEQ ID NO: 4 - DNA, 19 bp, Escherichia coli
  primer_bind (1)..(19): MB10.1rev qPCR primer
gtgctggctgcctgtttac

SEQ ID NO: 5 - DNA, 20 bp, Human papillomavirus type 18
  primer_bind (1)..(20): HPV18 104 fw1 primer for HPV
cagatccttatggggattcc

SEQ ID NO: 6 - DNA, 19 bp, Human papillomavirus type 18
  primer_bind (1)..(19): HPV18 105 rev1 primer for HPV
gattgaggcacagtgtcac

SEQ ID NO: 7 - DNA, 22 bp, Human papillomavirus type 18
  primer_bind (1)..(22): HPV18 106p primer
ggcatttttggaatagggcagg

SEQ ID NO: 8 - DNA, 19 bp, Human papillomavirus type 18
  primer_bind (1)..(19): HPV5901f primer
gtttagtgtgggcctgtgc

SEQ ID NO: 9 - DNA, 20 bp, Human papillomavirus type 18
  primer_bind (1)..(20): HPV5994r primer
ggcatgggaactttcagtgt

SEQ ID NO: 10 - DNA, 18 bp, Escherichia coli
  primer_bind (1)..(18): ThrB-Fw primer for E. coli thrB
acattcagtctcaacaac

SEQ ID NO: 11 - DNA, 18 bp, Escherichia coli
  primer_bind (1)..(18): ThrB-Re primer for E. coli thrB
aatttgcttacccagttc

SEQ ID NO: 12 - DNA, 34 bp, Escherichia coli
  primer_bind (1)..(34): Beacon-ThrB primer
cgcgatcgttctgacggcagcttatcggatcgcg

SEQ ID NO: 13 - DNA, 97 bp, Escherichia coli
  gene (1)..(97): E. coli amplicon1 (ThrA)
gacggtagattcgaggtaatgccccactgccagcagtttttcgaccggatcgataacagtaacgttgtgaccgcgcgcttctaatacgccggccata

SEQ ID NO: 14 - DNA, 114 bp, Escherichia coli
  gene (1)..(114): E. coli amplicon2 (ThrB)
acattcagtctcaacaacctcggacgctttgccgataagctgccgtcagaaccacgggaaaatatcgtttatcagtgctgggagcgtttttgccaggaactgggtaagcaaatt

SEQ ID NO: 15 - DNA, 191 bp, Homo sapiens
  N_region (1)..(191): K-ras amplicon
tagtgtattaaccttatgtgtgacatgttctaatatagtcacattttcattatttttattataaggcctgctgaaaatgactgaatataaacttgtggtagttggagctgatggcgtaggcaagagtgccttgacgatacagctaattcagaatcattttgtggacgaatatgatccaacaatagaggtaa

SEQ ID NO: 16 - DNA, 106 bp, Human adenovirus type 18
  gene (1)..(106): HPV18 amplicon
gattgaggcacagtgtcacccatagtacctgccctattccaaaaatgcctagcaaaaagctgctcacgccgtaagcaaaaaaacatggaatccccataaggatctg

SEQ ID NO: 17 - DNA, 18 bp, Escherichia coli
  primer_bind (1)..(18): C-Thr 1325f primer
cccgcgccaatatcaaca

SEQ ID NO: 18 - DNA, 20 bp, Escherichia coli
  primer_bind (1)..(20): C-Thr 1485r primer
accgacgccaatcacaaaca

SEQ ID NO: 19 - DNA, 20 bp, Homo sapiens
  primer_bind (1)..(20): Kras-cdn12-fw  primer
tagtgtattaaccttatgtg

SEQ ID NO: 20 - DNA, 18 bp, Homo sapiens
  primer_bind (1)..(18): Kras-cdn12-re  primer
ttacctctattgttggat

SEQ ID NO: 21 - DNA, 19 bp, Homo sapiens
  primer_bind (1)..(19): Dusp3 fw3 primer
agatggttttgcccgcttt

SEQ ID NO: 22 - DNA, 20 bp, Homo sapiens
  primer_bind (1)..(20): Dusp3 rev3 primer
tgccacttagcagaagcaac

SEQ ID NO: 23 - DNA, 23 bp, Homo sapiens
  primer_bind (1)..(23): Polynucleotide portion of Dusp3 tp3-2 FAM Taqman probe
ccacctcatatgtgtgtgctgcc

SEQ ID NO: 24 - DNA, 14528 bp, Homo sapiens
gggggcgggggcgcaggtagaggcgtgggggagaaggattcacacctgaggtgcaataaggaaaggaaggccagaggaatctttcattgaagacagattgtttgaggacaagcagctcctgtgaagaggctgcccagatcctctggtattttaactgggcaatgaatcagcatgccccacctgcagagcctctgcaagtcctttgccacctgcctcaacttgcaagtcgctgtgtccatctgcagccgactgtcctttccatcatccatcatccgacacatgaatgcagctgctctgacagttttacaagccagacagaagccccctcaggaagggccctctctgatacctgcttcctaagtcagtttccttcagggcagatgaaaacagctgtggccattgttgggggtgatctatctctcccagcagagccggtagtgttgtgagaagctggccctccgcgccacctccccttgtctatgaccctccagcctccttttcccttgctctggaatgtggactgttaaccctctcatgaccagacgactgccttcttgcaatggacttgggagagagcagttctgatgcctgggttccttgagcaggtaggatggatgcttatagccccacctgctgttgggagcggctggaccgtctgcattaaacagaggcagtgggattcatccctggaacgcgtctgccacctgctggagacaaaaggaggggtgactgcaggatggcaagtctcaggactggacgtgatttcctttcctttcctttccttatttggaagtgaagtaatattaaaaggaaaaagaagaatccagtggacttgaacctctaaatgatccacacccctctgaatggctcagcgagaacctgctgtgacatcttctgctgtttcatttaatgttaagtcattgacagctgtttatttttactcagtccacaaacttgtcattgttcacagtattccctggaattaaacccccagggttttagctgattcctattgtgagtagtttaggttatttccaattttttttcctatttccagcagggttgctatgaacatccttgtacggctgaaattttttttttttctttttttggcagattctctctgtggcccaggctgcagtgcagtggcacaatcttggctcactgcaacctccacctcctgggttcaagcaattctcctgcctcagcctcccgagtagctgggattacaggaatgcaccaccacgcccggccaattttgtatttttagtagagacgggggtttctccatgttactcaggctggtctcgaacttctgacctcgggtgatctgcccaactcggcctcccaaggtgctggggattagaggcatgagccacaatgcccggcctcagagtaattttttaaattaaaattttaaaatgtggatataattataaatttaaatatacttataagaaataaaagcccgggcaacatggtgaggcctagtctctacaaaaaatttaaaaattagctgggcatggggtcgcacgcctgtggtcttagctacttgggaggctgaggtgggaggttcacttgaggttgaggtcgaggctgcagtgagccatacttgggccactgcactccagcctggttgacagagtgagaccccgtctcaaaaaataaaaataaaaaaaagaaaatgcagactccgtgtatcctttatccagtttcccacaacaataacaccttgcgaaactataggacaatatcacaactaggatattgatattgacacaatttaccaatcttacccacatctcccgtggcttaacctctactgtgtgcgtgcacacgcattcacgtgtgtgtatacttagttctatgcaatcttgtcacgggtaaatttggggatccaccacagtcaagataaagcacagctctgtgaccacaagtctttctcctgttgcccacctccttccctccttttccctccctcccacaactaacccctggcaactactcatctaatctccatttctgtcattttttttttcacttcaaaattgttacataaatgcgaccaggtgcggtggctcactcatgtaatcccagcactttgggaagccaaggcaggcagatcacttgaggtcaggagttcgagaccagcctggccaacatggcgaaaccctgtctctactaaaaatacaaaaattagctgggcatggtggcacgcacctgtaatcccagctatttgggaagctaaggcaagagaatcgcttgaactcaggaggcggaagttgcagtgagctgagatcgcgccactgtgctccagcctgggtgacagagtgagactgtctcaaaaaaaaaaaaaaggttatataaatggaatcaattagtatgtagcctttggggatttttttttcactcagcattatttccattatccaagttgtacatatcagtaacatgttcctttttcttttctttttttttttttggctgagtagtattccacaaagtttaaaaaaacaaaacaaaactttagagttatttctggaagtgaatgctgtgtctgagggagtgtgaagagtttggtggtctgatgagggtattgcagggctgttttccagaaaactcagcccagtccccgccctcacctgcaaaatagaggctcccataggtggtactttgatgaggctgccgtaactaagtaccacaaattgggtggcataaacaacagaagtcgtctcacagagctggaggttaggagtgcaagttcaagacattggcagagttggttccttcgaggacagtgaggaaggccttttacctgccttctgctggctgctgacaagctgtggcattcactggcttgcagaagtgtcacccccaatccctgccttcatcttcacatggtgttctctctgtgttcgaattttcccttttttctaaggaggtcaggcatattagattaggcccagcctaacgacctcatcttaacgagttacatctgtaatagccctatttccaaataaggtcacattctcaggtactgtgacttaggacttcaatatatgcatttgggaggaatgcagttcaacccataaataagactgtcaacactgggtttgggatgttgatttttttttttttttttttttttttttttgagacagagtctcgctctgtcacccaggcgggagtgcagtggtgtgatcttggctcatataacctccacctcctgggttcaagcagttctcctgcctcagcctcccgagtagctaggactacagactcccgccaccacacccagctaatttttgcattttttttgtttgttttgtagagatggggtttcgccatgtcggccaggctggtcttgaactcctgacatcaggtgttcccacaatcccataaagtgctgggattgcaggcgggagccaccgcacccagccgatttttttaaacattgaatttaacagttgaaacttaatttccagaaaagctgcttttccatgtgattatttaccagcttttgtttctgtcgagttgcttcttccgatgttcactcgccaaacgtttaataaagcaagggggacacgcactccctctccaggagctcgcataccatggaagaaataatttccgcatccaaacaactccactaccagatggaaggtgatcaatgccactgaaaaaaaggttcagatgcttttttctaaaaaaaactttattttttttctggagcacttttaggttcacagcaaaactgagtggatggtacagagatttctcatttatgtcctgtgcccacacatgtacagctgcccccgttatcaacatcccgccaccagagtggtgcatttgctatgattgatgagcctacatgacacatcattatcacctgaagtccatggtttacatcacagcactagtgttgtacatcctatggctttggacaaatgtataatgacatacatctaccattatagtatcatacagatgggcagtattttcattgtccaaaaaaactatctgctctgcctattcatccctccccgactttccccaacccctggcaaccactgatctttttactgtacctttatttttgccttttccaggatgtcatatagagttggaatatacccatacatagtcttttcagattggcttctttcagttagtaatattcatttggggttcctccatgtcttttcatggcatgaacagcttattttttttttttagcactgagtaatactccattcgtcttgatgtatcacggtttatctagtcacctactgtcatctactgaaggacatcttggttgctttcaagctctggcaattattaatagaggtggtataaacattttgcacaggttttttgttttgttttgtcttaagacggagtcttactctgtctcccaggctggggtgcagtgccgtgatctcagctcactgcaacctccgcctcctgggttcaagtgattctcctggctcagcctcccgagtaggtgggattacaggtgagcaccaccacacctggctaatttttgtatttttagtagagaaggggtttccccatgttggccagtatggtctcaaactcctaacctcaagtgatctgcccacctcagcctcccaaagtgctgggattacaggcatgagccaccatgcccagctgtgtgcaggtttttatacgaacgttaagttttcaaatcatttgaataaataccaaggagcatgactgctggattgtgcaataaaagtatgtgtagttttgcaagaaactaaactgcaaactgtcctccaaagtggctgtaccattttgcattccccactgaaacaaagagttcctgttgttccacatcctcaccagatgcattttttcaaaaggacaattttcttatgggccttcaaaggagagaacaatctctttcccctggggaggatctgggatccttatggtaagatgtggcatttggaccagactttgaatgacaggccaaatttggaaagtatattatgctcctttgactccttgggatcatagaatctttgatctggaaggactctcaaaggtcatccggtttcattctctacttggttctggaggaggcccctatctctaattaatggaaactgaggattctccttattggctgcattttaaaacagattttgctcccacttgtaggtggtaaaaaggaaatatctggattaggagggcaaacttctgcttttaggcagtaccctgcattgagggatgtccaaatcaccttgtctttatttacacatccatacacaatggaatgctatgtagctgttaagatgaagggggtagaacaataaaaacaataaccataatataagctaagcaaaacaaacaacaaagcagagatatctctgtatatacacacgtatgcacatatgtgtgcttatatatgcttgacattttcctttaaggatatgatgcttatggggagacagattgaaggagcaagtgactcacttttccgtataagccttttgcattgtttaagtgtattactatgtacatatagtattatttttaatgaaaaattttttaaaaattatacttaaaaacttttacctgttttatattttagtgctctgccttaagattttgtgtagaaccataaagattacattgtcagagtcttgacaaataggaagcgagtccaattgcttcatgtgatagagggaatgggaacctcgagaggctttctctgcccagacttctgtctgggaggaaaaggcaactactttctctaaggttttttattcaaaggaacatagcaccaatagtggaatttaaggcatctgggggaaggggatatgtttagggactgttcatttgcaggatcactcaaatctcaaaatgtcacccagtcatcacgtgaggctaccttgagatgaacaccctagtcccctgctttcttagaagcacaaaccttacctccttcattcaggaccattatggccattctacctaagaatattcctaccagaacatttctggtactggaaaggtgttcatcaatatctactgcataaacagtgccatcatggaacctataactagctcagaacggctatgttttagatgattatttttaaaaagttagaaatcgcaaatataaaagctaagcccaaacaaaaaaagctaagcataaaaacgtaaaagaataccaactgtgataagaaggacaaaaaaacaatacctttgtaatgtaagacatttattttggctaaagttctggtgttttaacactgatttgtgatacaacggacattaaacttccttttaaaaagaaaaaaacaatttggtagctctcccttttctgtccagaaaaattcactctttcataatcaaattaccctaaaatttggtggcgttaagaggcaacaaaagttaagcttccaacgaatctgttctctcaaccggaaatgtcttctatttccaatcaggataaaaccttgacttacttgcaaggactatcacggttagcccttcagtgattcctgacaccagttctgtgaaaaagaaaatttcctgcgagaaaagctcatgtcttcatattgaagatcagtacttttttttttttcctttaaaacagtagcatcttaacttgtggcacaaaaggcaccaacattccctttccaaaccatccatcaccatgggtggaaggcagcgccacctgctgcccatcatattatggctcacatacccataatttccttgcggtgctgaattccaagtggggattattagagacccctcagagccaaaaggggaccttagaggtcttctagatgagtcccctcatttgtaggtggtggtttctggataactcagagtggcagggacacagacgagcctgtggaaaggtatactgctttaagattgagaagaaaaccatttggcgctctaattttgcctggatggtgctctgtcagtcaaagaaagggaacaggtctggggagggggtaagggcaccctgagttcctgttccatcacttcccaggcagtagaaggctgtccaggaacagctcccatccgcagctgggcatgtgttggctcttacacaagagactttaattttacttgaagaactaagagctaaatcttgttaagtaaatacggggtttcaggggtgaaggactatcaagaaatcccaagttatcagcataaaagtagtcccaaagtaaaggcagtaattctcccaatggccttttctccctcatgcccccacagagactttcgagaggtcctagttagccagccacaccaacctgctgtgttcgcgtaagtagctgtgcctgtcccatggggtgaccactgcctggtcatgggaggggagccccagccccagctccctagccttttccaggagcagagcagaaagctctacttcggggtgctacatcccacctggagaaagagctgcacattctagcctatgagggacccacccttttcacttgcttctccggggctggattgagggtaagtgcagtacacctggagatcccagggagcccccttcttgagaaagagtatcgtatgaaagaatccagcttcagggagcagcaaacccaaaatcttgcccagctccaccttatggagctggacaaccctgggggccaggcccttaatcattctgaacctcagttccttttttttaaaaaaggtcacaatacaagaacaagctctactaactttacagggttactgtgaggctcaagttagattaagttggaaggctacctagaagctgtgcagtgaggtacccagtttagaggatggccatttcacttaggtgggtttatctggacacctttttcactatctggagaagaagacacatactggttgttcagggctgctgtggtcacagagaaaagcggacagcaaatgaccaggctgggcagggctgcttctgtgtgatcagagaccttcacagccgggagtgaggccttacgccacacctgcctctccgtgtcccagccaggagctcctggccaactctgaaaaaggcacattccctaccttggcatattaacactgcctgaatttaaatgtaaaactgagttgtaaatagtcaacaaaagtccctgatatttctttcgttttaggtaagactccttcacaaggccttgcgagtgatcctaccatgaattcagtcttctgggagcgtgacacacccaccagaacaatgccctatatatatttggtgctcaaaaagtgtttaatttcttaaacttttatcagacacctatgtgcaaggtgctgggggcatggctgaggaccttctctttgcccagagtgaccctgaagataaatagcatcacaatcactttccataataacaataacgtaaaatcctaacaagactgtatttaaaacaaaactcttatattctggcaaatgtgcatacacatgtgagggctggtgcattccaatatcatccttagaaagtcttttgaaaggtttatcgtgtttgggtttttttgctctaccaccaataaaggatccatttggacactccaccatgtctcatgtctgcctggctgagtcacttcagggatcccgtgctggcaccagagagctgtaagagccacctgcaatgggcagggtgtgtgcctgggacctttcacttccctgcttgtcttctggccgcgtttctgagaggcacgccccccacacacatccatgcacacacgctgtaattggccaacttcctccttctgttcttggaatagcaaccgagacaaaaagcagttagcacgagtggcttgggcttgccaacactacaattcaggacaaaacccttgtaattctccaaatggtggggtttttaaataggttggacttcaactccctgttttctaaaaaagaaaaaaaaaagcatgcccaaggcatcactcttctcaaaaacgaagtgactgagataagatcgaagggaaatattccagagcagcagattctgaactcaaggcttccaaagattcacattttgaaaactctatggatttaggagggttctccaggtttgcccacaaggcctctttgtgtagggaccattcatcctaaggaaatcattcaaatgcagccttgctgtgggaatctccatccactaataactgacggacacccccaccccagcttcggacctcaagacgtgagagggttgcctatgcacagggtgtggaaggctgtggggacagtgcggggcacagacgtggtggggagagtggcctgcatttgcatagttcctttactagggctcaaggtgttgaggtccacactcaagagaggattcgggagttggggaagggaggtcatgagggacctctgtgagcatcttaggccttacacttccacacacctcctgccgtgggccatcgggaagcatgcaggccacaggccttccccctctgagcccccatctcagggaaaagacatcataagttacagaaacaggacaactggggagcaaggacgccccccttggcaagcttctttatgtgctccccagggtggggaaagtggcccaggactgtgttgggacacacttgtagacaagtgccttgtgatgctgggagcagggtacagtgtgtttcctaaacatggcagctcgggacacctttgcccacggcctcccccacggacctctcgagcagaggcggtgggggtgccctagggtttcaacttcccctccttggctagtctgtcattgagctggcagagctgggccaggaagccatcgttggggccgatctcacggttctgcctcacgatgctcagggcagacttgacgtccatcttctgccgcatcatgaggtaggcgataactagcgttggggagcggctataaccttcccggcagtggacgagcacccggcctgtaagaaacaggggagacgtggtgagctgggggcgtcccatcacaccatggcgttggtcaagactcttccgtgaagtgccacttaaaagcacaatgtcacgccactgtgtgcctgccagaatggctaaaatgaaaaggatggaaaacccaaagtgctggtgaagatatggggcaactggaactcttctgcgtggctgggggaggtgaggcgtgaattggcacaaccacttcggaaagctgtgcggcacggcggtatctcctcaagctgaacacgtgcatcccctctggcccagcaatcccactcccaggcccaggtccaatagagatacgcattcacattcacgaacatgggccagaatgttcacaggcaacactgcacatcatggcccacagttagaaacccccaaaggcccatccacagtagaaaggacaaatacaaagaatgaccagactgccacttagcagaagcaacacggaggcagcacacacatatgaggtggatgagcccacagagtaggaaagcgggcaaaaccatctgtgctgtcagaagcctgcaaggggctgggcacagtggctcacgcctgtaatcccagcactttgggaggccaaggcaactggatcacaaggtcaggagttcgagaccagactggccaacatagtgaaatcccgtctttactaaagatacaaaaaaatagctgggtgtggtggcgcgagcctataatcccagctactcaggaggctgaggccagagaattgcttgaacccaggaggcagaggttgcggtgaggtgagattgtgctgagattgtgctccagcctgggtgacagagcgagactctgtctcaaaaaaaaaaagaagcccgcgtggcagaggccctgggagctggggatgggggtggtggagcatagagactgggggtgctttccagggtgctggtagtgttttgtttctttttttttgagatggagtttccttcttgttgcccagggtggagtgcagtggcgcgatctcggctcacttcagcctccgcctcctgggttcaagcaattctcctgcctcagcctcctgagtagctgggactacaggcgcatgccaccatgcccagctaatttttttgtatcttttagtagagatggggttattttaatatagtgtgtgtgtgcgtgtatatatatatgtgtatgtgtgtgtgtgtgtgtgtgtgtatgtgtgtgtatatatatatatataaatagacaccatctctcaatatccacagggcagattggctccaggacctcctgccgatacccaaatccacagatgctcaagtccctgattataaaatgacatcatatatgcaaataacctctgcacagcacatcctcccctatactttaaatcatctccagatgacttatgatacccaagacaatgtaaacatttattagattatatcatctagagaataatgacaagaaaaaaaatctgtacatgttcagtacagacataacatctttttatgttgtttttaatatttttcagactgcggttagttgaatccacagatgtggaacccacggatatggaggaccgactgtatattctattggttctgttttttctagagaatcctgaccaatacactggttattaactcatgatccacctaacctcaaggtgcctcagttttcttatctggccaatagtacccattgcacaaggtggttagaagattaaaggagaggacacatgaatcctctaggttagcacctggcatccatgtgcactcaataaatgttacccaatactgggcatcctctggtagcacctagtacaccctcaactacagcagccctggtcctgtgtcattgccagacatgcgcagattgacttttctctcccagaggacgaattctttaagagcaagaaatggccggacacagtggctcacacctataatcccaacactttgggaggtcgaggtgggcggatcccctgaagtcaggagttcgagaccatcctggccaacatggcgaaaccccgtttctactaaaaatacaaaaaattagctgggcatggtggcacatgcctgtaatcccagctactcagaaagctgaggcaggagaatcacttgaacctgggaggtggagggtgcagtgagctgagattgagccactgtactccagcctgggtgacaagagcgagactccgtctcaaaaaaaaaaaaaaaaggcaagaaatgtggggcattgatttttggatgcgttacaatctctagcatacactatgtgctcaataaatatttgctgactagctgagtgaattattacctactaacacctctataaggccattgtttggcaaggaatctgctagcccagagtccaacagagtctcttctgctcctatcaccctacccccaaaacaccactctattttcccaatgccttccaaatcaggaagcaggagtcctccactttcttgcccattcaccctccggcctgtatgcccgaaatattcagagtggggcttcccctgccccaccctaggaatgagaccctctgcagagcagccaccttaccatctagaacatactctgcatgcccagtgcacacagagcctactgggaaaggggccagttcaacctcccattcctctaggctcagcccagatgccacctcctccatgaagctgttttcccagctagaagtgactgctccctcttgagtaccctcagccatcccacccagctctcagtgatgggtccctgggccccacacactgttggaggccagcatgtttctgttgactcacttcgccactcattcttagaagcatttatacttggcattagagcccatggaattcttcatcacttgctcattcatcatttgcagtgtacctactatgtgcctgatgctacatcaggtgctaaggagacagacaaggaacaaagtagacccagcctgagggcaggcttcatggaagagaggacatcatgccaaggacaaggtggagtttgccagaggaaggggtagggagaggcagagagaacttttcagactaaagacccagcacacctggactgagacaggtcaaaaaaagggcgtgttcctagttgtttggaaagaggaaacaaagtcagagagcttgaaattccctgaatgaataaccaattgctattatacgagaacaacaaaatccttccccttcgcccagcctatgtttacacagggtgaggaactcagtacagctggagtggaggaggtgagcagggttggggggtgacagtgaccaggaaggaccatgaggggcctgtcagcaaagtctgcagatactccgcagtaaagcttctctctgagccctgagcgttcactgtccagtggtctagaaaattctgtttactggaaatcattcagacagtgagcctgctgggcccaagagtcatcagtgtagtacagccaaggctgttcacacctcatgggggtcccctccgctgggagggtttggggtggggagagaggaagaggtaaagggaggagctgagagaaacagctaaaagcagaaagggagaaagggcaagtggcccagcctgctcagctgatgtctgctttgtggccttctagggtttcttgctggaatgccttggtgactgccagcgccttggtagttctccttcagtcttatcttatatttgggggctgcaggaagtgtttcgtaagtggctggaagatttggccaggggggctgtggtttgctgactgccaacctaagctgaccgcagctaccccttttctccttgccaggcaatcacgtgaatctctagccaatgagatgtgaggggtatttctgggaaatgttttacttgttcttaaagagagagactgggcatggtggcacgtgcttgtagtcccagctactcaggaggctgaggtgagaggactgcttgagcccaggagttggagaccagtctagacaacatagcaagaccctgtctctttaaaaaagagagagagagtggccaggcgcggtggctcatgcctgtaatcccagcactttgggaggcagagggaggcggatcacctgaggtcaggagttggagaccagcctgaccaacatggtgaaaccccatctctactaaaaatacaaaattagccaggcgtgggggcgcatgcctgtaatcccagctacttgggaggctgaggcgggaggctgaggcaggagaatcgcttgaacctgggaggtggaggttgcggtgagccaagatcgcgccattgctcttcagcctgggcaacaagagtgaaactccatctaaaaaaaaaaaaaaaaaggagagagagaagaggaaaaaaagagtgggaagagatggctgcagggcctcatctgctgtactttgtcctgcttggatgtggtgactggatcccatcttgggaccatgacgggagcacccaacactgaggtggcagaagagagaaagggaaagggcctggtccagaggccaccatggagctgctgaatcaagcagccccttaatcaaccagaccccatgctccttcacctcaggacttcttgccatgcacattaacacattaacacatcttcctcatcgttacagctgtttgca